European Patent Specification EP 4 337 788 B1, published October 30, 2024. Title: SPATIAL ANALYSIS OF A PLANAR BIOLOGICAL SAMPLE. Applicant: MOLECULENT AB. The sequence listing filed with the application follows.

SEQUENCE LISTING (5 sequences)

SEQ ID NO: 1 - DNA, 36 bp, artificial sequence
  synthetic oligonucleotide
tttuuucgtutacgaccucuaaggccacgauagcgt

SEQ ID NO: 2 - DNA, 36 bp, artificial sequence
  synthetic oligonucleotide
atgcuaaccgcagaccactaggcgaatacgtttttt

SEQ ID NO: 3 - DNA, 20 bp, artificial sequence
  synthetic oligonucleotide
cggttagcatacgctatcgt

SEQ ID NO: 4 - DNA, 60 bp, artificial sequence
  synthetic oligonucleotide
ggccttagaggtcgtaaacgtttgaagcaatccgtgggcgggcgcaaacgtttgtcgaca

SEQ ID NO: 5 - DNA, 60 bp, artificial sequence
  synthetic oligonucleotide
aatgtttcgcgtgcatccggctccaccggatttgcagcttcgtattcgcctagtggtctg